European Patent Application EP 4 378 944 A1, published June 5, 2024. Title: Compound having photocleavable site, conjugate and screening method using the same. Applicant: CHUGAI PHARMACEUTICAL CO.,LTD. The sequence listing filed with the application follows.

SEQUENCE LISTING (7 sequences)

SEQ ID NO: 1 - protein, 156 aa, synthetic construct
  REGION 1..156: note = eSrtA
MQAKPQIPKDKSKVAGYIEIPDADIKEPVYPGPATREQLNRGVSFAEENESLDDQNISIAGHTFIDRPNYQFTNLKAAKKGSMVYFKVGNETRKYKMTSIRNVKPTAVEVLDEQKGKDKQLTLITCDDYNEETGVWETRKIFVATEVKLEHHHHHH

SEQ ID NO: 2 - protein, 207 aa, synthetic construct
  REGION 1..207: note = KRAS4Bwt(C_FLAG-Sor-His)
MTEYKLVVVGAGGVGKSALTIQLIQNHFVDEYDPTIEDSYRKQVVIDGETCLLDILDTAGQEEYSAMRDQYMRTGEGFLCVFAINNTKSFEDIHHYREQIKRVKDSEDVPMVLVGNKCDLPSRTVDTKQAQDLARSYGIPFIETSAKTRQGVDDAFYTLVREIRKHKEKMSKDGGSSDYKDDDDKGGSSLPMTGGGGSSHHHHHHHH

SEQ ID NO: 3 - protein, 529 aa, synthetic construct
  REGION 1..529: note = NusA-SrtAHis
MNKEILAVVEAVSNEKALPREKIFEALESALATATKKKYEQEIDVRVQIDRKSGDFDTFRRWLVVDEVTQPTKEITLEAARYEDESLNLGDYVEDQIESVTFDRITTQTAKQVIVQKVREAERAMVVDQFREHEGEIITGVVKKVNRDNISLDLGNNAEAVILREDMLPRENFRPGDRVRGVLYSVRPEARGAQLFVTRSKPEMLIELFRIEVPEIGEEVIEIKAAARDPGSRAKIAVKTNDKRIDPVGACVGMRGARVQAVSTELGGERIDIVLWDDNPAQFVINAMAPADVASIVVDEDKHTMDIAVEAGNLAQAIGRNGQNVRLASQLSGWELNVMTVDDLQAKHQAEAHAAIDTFTKYLDIDEDFATVLVEEGFSTLEELAYVPMKELLEIEGLDEPTVEALRERAKNALATIAQAQEESLGDNKPADDLLNLEGVDRDLAFKLAARGVCTLEDLAEQGIDDLADIEGLTDEKAGALIMAARNICWFGDEAGGSSDYKDDDDKGGSSLPMTGGGGSSHHHHHHHH

SEQ ID NO: 4 - protein, 254 aa, synthetic construct
  REGION 1..254: note = GST-SrtAHis
MSPILGYWKIKGLVQPTRLLLEYLEEKYEEHLYERDEGDKWRNKKFELGLEFPNLPYYIDGDVKLTQSMAIIRYIADKHNMLGGCPKERAEISMLEGAVLDIRYGVSRIAYSKDFETLKVDFLSKLPEMLKMFEDRLCHKTYLNGDHVTHPDFMLYDALDVVLYMDPMCLDAFPKLVCFKKRIEAIPQIDKYLKSSKYIAWPLQGWQATFGGGDHPPKSDGGSSDYKDDDDKGGSSLPMTGGGGSSHHHHHHHH

SEQ ID NO: 5 - protein, 273 aa, synthetic construct
  REGION 1..273: note = sfGFP-SrtAHis
MVSKGEELFTGVVPILVELDGDVNGHKFSVRGEGEGDATNGKLTLKFICTTGKLPVPWPTLVTTLTYGVQCFSRYPDHMKRHDFFKSAMPEGYVQERTISFKDDGTYKTRAEVKFEGDTLVNRIELKGIDFKEDGNILGHKLEYNFNSHNVYITADKQKNGIKANFKIRHNVEDGSVQLADHYQQNTPIGDGPVLLPDNHYLSTQSVLSKDPNEKRDHMVLLEFVTAAGITHGMDELYKGGSSDYKDDDDKGGSSLPMTGGGGSSHHHHHHHH

SEQ ID NO: 6 - RNA, 74 nt, synthetic construct
  misc_feature 1..74: note = tRNAGluCUA
  source 1..74: mol_type = other RNA
gtccccttcgtctagaggcccaggacaccgccctctaacggcggtaacaggggttcgaatcccctaggggacgc

SEQ ID NO: 7 - RNA, 75 nt, synthetic construct
  misc_feature 1..75: note = tRNAfMetCAU
  source 1..75: mol_type = other RNA
ggcggggtggagcagcctggtagctcgtcgggctcataacccgaagatcgtcggttcaaatccggcccccgcaac